European Patent Specification EP 3 906 065 B1, published April 30, 2025. Title: Minimization of systemic inflammation. Applicant: Ascendis Pharma A/S. The sequence listing filed with the application follows.

SEQUENCE LISTING (29 sequences)

SEQ ID NO: 1 - protein, 132 aa, Artificial Sequence
  aldesleukin mutein
PTSSSTKKTQLQLEHLLLDLQMILNGINNYKNPKLTCMLTFKFYMPKKATELKHLQCLEEELKPLEEVLNLAQSKNFHLRPRDLISNINVIVLELKGSETTFMCEYADETATIVEFLNRWITFSQSIISTLT

SEQ ID NO: 2 - DNA, 20 bp, Artificial Sequence
  Ubb forward sequence
gtctgaggggtggctattaa

SEQ ID NO: 3 - DNA, 20 bp, Artificial Sequence
  UBB reverse sequence
gcttaccatgcaacaaaacc

SEQ ID NO: 4 - DNA, 20 bp, Artificial Sequence
  Ccl2 forward sequence
cagctctctcttcctccacc

SEQ ID NO: 5 - DNA, 20 bp, Artificial Sequence
  Ccl2 reverse sequence
tgggatcatcttgctggtga

SEQ ID NO: 6 - DNA, 20 bp, Artificial Sequence
  Ccl3 forward sequence
ccagccaggtgtcattttcc

SEQ ID NO: 7 - DNA, 20 bp, Artificial Sequence
  Ccl3 reverse sequence
aggcattcagttccaggtca

SEQ ID NO: 8 - DNA, 20 bp, Artificial Sequence
  Ccl4 forward sequence
tctgtgctaaccccagtgag

SEQ ID NO: 9 - DNA, 20 bp, Artificial Sequence
  Ccl4 reverse sequence
ctctcctgaagtggctcctc

SEQ ID NO: 10 - DNA, 20 bp, Artificial Sequence
  Ccl5 forward sequence
tgccaacccagagaagaagt

SEQ ID NO: 11 - DNA, 20 bp, Artificial Sequence
  Ccl5 reverse sequence
agatgcccattttcccagga

SEQ ID NO: 12 - DNA, 20 bp, Artificial Sequence
  Csf2 forward sequence
ctgcgtaatgagccaggaac

SEQ ID NO: 13 - DNA, 20 bp, Artificial Sequence
  Csf2 reverse sequence
tctctcgtttgtcttccgct

SEQ ID NO: 14 - DNA, 20 bp, Artificial Sequence
  Cxcl1 forward sequence
ttgtatggtcaacacgcacg

SEQ ID NO: 15 - DNA, 20 bp, Artificial Sequence
  Cxcl1 reverse sequence
acgagaccaggagaaacagg

SEQ ID NO: 16 - DNA, 20 bp, Artificial Sequence
  Cxcl2 forward sequence
ctacatcccacccacacagt

SEQ ID NO: 17 - DNA, 20 bp, Artificial Sequence
  Cxcl2 reverse sequence
tgttctactctcctcggtgc

SEQ ID NO: 18 - DNA, 20 bp, Artificial Sequence
  Cxcl10 forward sequence
gccgtcattttctgcctcat

SEQ ID NO: 19 - DNA, 20 bp, Artificial Sequence
  Cxcl10 reverse sequence
gataggctcgcagggatgat

SEQ ID NO: 20 - DNA, 20 bp, Artificial Sequence
  Il1b forward sequence
actcattgtggctgtggaga

SEQ ID NO: 21 - DNA, 20 bp, Artificial Sequence
  Il1b reverse sequence
ttgttcatctcggagcctgt

SEQ ID NO: 22 - DNA, 20 bp, Artificial Sequence
  Il6
ttcttgggactgatgctggt

SEQ ID NO: 23 - DNA, 20 bp, Artificial Sequence
  Il6 reverse sequence
caggtctgttgggagtggta

SEQ ID NO: 24 - DNA, 20 bp, Artificial Sequence
  Il10 forward sequence
acctggtagaagtgatgccc

SEQ ID NO: 25 - DNA, 20 bp, Artificial Sequence
  Il10 reverse sequence
agggtcttcagcttctcacc

SEQ ID NO: 26 - DNA, 20 bp, Artificial Sequence
  Il18 forward sequence
ggacactttcttgcttgcca

SEQ ID NO: 27 - DNA, 20 bp, Artificial Sequence
  Il18 reverse sequence
accctccccacctaactttg

SEQ ID NO: 28 - DNA, 20 bp, Artificial Sequence
  Tnf forward sequence
tgaggtcaatctgcccaagt

SEQ ID NO: 29 - DNA, 20 bp, Artificial Sequence
  Tnf reverse sequence
ggggtcagagtaaaggggtc